European Patent Specification EP 3 659 440 B1, published January 18, 2023. Title: PLANT GROWTH PROMOTING MICROORGANISM AND ENZYMES FOR SOIL BIOGENIC CYCLES. Applicant: BIO-ILIBERIS RESEARCH & DEVELOPMENT S.L,. The sequence listing filed with the application follows.

SEQUENCE LISTING (3 sequences)

SEQ ID NO: 1 - DNA, 16 bp, Bacillus sp. BIRD-6
agagtttgatcctggc

SEQ ID NO: 2 - DNA, 16 bp, Bacillus sp. BIRD-6
taccttgttacgactt

SEQ ID NO: 3 - DNA, 1148 bp, Bacillus sp. BIRD-6
catgcaagtcgagcggacagatgggagcttgctccctgatgttagcggcggacgggtgagtaacacgtgggtaacctgcctgtaagactgggataactccgggaaaccggggctaataccggatggttgtttgaaccgcatggttcaaacataaaaggtggcttcggctaccacttacagatggacccgcggcgcattagctagttggtgaggtaacggctcaccaaggcgacgatgcgtagccgacctgagagggtgatcggccacactgggactgagacacggcccagactcctacgggaggcagcagtagggaatcttccgcaatggacgaaagtctgacggagcaacgccgcgtgagtgatgaaggttttcggatcgtaaagctctgttgttagggaagaacaagtaccgttcgaatagggcggtaccttgacggtacctaaccagaaagccacggctaactacgtgccagcagccgcggtaatacgtaggtggcaagcgttgtccggaattattgggcgtaaagggctcgcaggcggtttcttaagtctgatgtgaaagcccccggctcaaccggggagggtcattggaaactggggaacttgagtgcagaagaggagagtggaattccacgtgtagcggtgaaatgcgtagagatgtggaggaacaccagtggcgaaggcgactctctggtctgtaactgacgctgaggagcgaaagcgtggggagcgaacaggattagataccctggtagtccacgccgtaaacgatgagtgctaagtgttagggggtttccgccccttagtgctgcagctaacgcattaagcactccgcctggggagtacggtcgcaagactgaaactcaaaggaattgacgggggcccgcacaagcggtggagcatgtggtttaattcgaagcaacacgaagaaccttaccaggtcttgacatcctctgacaatcctagagataggacgtccccttcgggggcagagtgacaggtggtgcatggttgtcgtcagctcgtgtcgtgagatgttgggttaagtcccgcaacgagcgcaacccttgatcttagttgccagcattcagttgggcactctaaggtgactgccggtgacaaaccggaggaaggtggggatgacgt